European Patent Application EP 4 368 200 A2, published May 15, 2024. Title: ANTICANCER COMBINATION THERAPY. Applicant: BOEHRINGER INGELHEIM INTERNATIONAL GMBH. Application EP. The sequence listing filed with the application follows.

SEQUENCE LISTING (20 sequences)

SEQ ID NO: 1 - protein, 446 aa, synthetic construct
  REGION 1..446: note = HC of PD1-1
EVMLVESGGGLVQPGGSLRLSCTASGFTFSASAMSWVRQAPGKGLEWVAYISGGGGDTYYSSSVKGRFTISRDNAKNSLYLQMNSLRAEDTAVYYCARHSNVNYYAMDYWGQGTLVTVSSASTKGPSVFPLAPCSRSTSESTAALGCLVKDYFPEPVTVSWNSGALTSGVHTFPAVLQSSGLYSLSSVVTVPSSSLGTKTYTCNVDHKPSNTKVDKRVESKYGPPCPPCPAPEFLGGPSVFLFPPKPKDTLMISRTPEVTCVVVDVSQEDPEVQFNWYVDGVEVHNAKTKPREEQFNSTYRVVSVLTVLHQDWLNGKEYKCKVSNKGLPSSIEKTISKAKGQPREPQVYTLPPSQEEMTKNQVSLTCLVKGFYPSDIAVEWESNGQPENNYKTTPPVLDSDGSFFLYSRLTVDKSRWQEGNVFSCSVMHEALHNHYTQKSLSLSLG

SEQ ID NO: 2 - protein, 218 aa, synthetic construct
  REGION 1..218: note = LC of PD1-1
EIVLTQSPATLSLSPGERATMSCRASENIDTSGISFMNWYQQKPGQAPKLLIYVASNQGSGIPARFSGSGSGTDFTLTISRLEPEDFAVYYCQQSKEVPWTFGQGTKLEIKRTVAAPSVFIFPPSDEQLKSGTASVVCLLNNFYPREAKVQWKVDNALQSGNSQESVTEQDSKDSTYSLSSTLTLSKADYEKHKVYACEVTHQGLSSPVTKSFNRGEC

SEQ ID NO: 3 - protein, 446 aa, synthetic construct
  REGION 1..446: note = HC of PD1-2
EVMLVESGGGLVQPGGSLRLSCTASGFTFSASAMSWVRQAPGKGLEWVAYISGGGGDTYYSSSVKGRFTISRDNAKNSLYLQMNSLRAEDTAVYYCARHSNPNYYAMDYWGQGTLVTVSSASTKGPSVFPLAPCSRSTSESTAALGCLVKDYFPEPVTVSWNSGALTSGVHTFPAVLQSSGLYSLSSVVTVPSSSLGTKTYTCNVDHKPSNTKVDKRVESKYGPPCPPCPAPEFLGGPSVFLFPPKPKDTLMISRTPEVTCVVVDVSQEDPEVQFNWYVDGVEVHNAKTKPREEQFNSTYRVVSVLTVLHQDWLNGKEYKCKVSNKGLPSSIEKTISKAKGQPREPQVYTLPPSQEEMTKNQVSLTCLVKGFYPSDIAVEWESNGQPENNYKTTPPVLDSDGSFFLYSRLTVDKSRWQEGNVFSCSVMHEALHNHYTQKSLSLSLG

SEQ ID NO: 4 - protein, 218 aa, synthetic construct; identical to SEQ ID NO: 2
  REGION 1..218: note = LC of PD1-2

SEQ ID NO: 5 - protein, 446 aa, synthetic construct
  REGION 1..446: note = HC of PD1-3
EVMLVESGGGLVQPGGSLRLSCTASGFTFSKSAMSWVRQAPGKGLEWVAYISGGGGDTYYSSSVKGRFTISRDNAKNSLYLQMNSLRAEDTAVYYCARHSNVNYYAMDYWGQGTLVTVSSASTKGPSVFPLAPCSRSTSESTAALGCLVKDYFPEPVTVSWNSGALTSGVHTFPAVLQSSGLYSLSSVVTVPSSSLGTKTYTCNVDHKPSNTKVDKRVESKYGPPCPPCPAPEFLGGPSVFLFPPKPKDTLMISRTPEVTCVVVDVSQEDPEVQFNWYVDGVEVHNAKTKPREEQFNSTYRVVSVLTVLHQDWLNGKEYKCKVSNKGLPSSIEKTISKAKGQPREPQVYTLPPSQEEMTKNQVSLTCLVKGFYPSDIAVEWESNGQPENNYKTTPPVLDSDGSFFLYSRLTVDKSRWQEGNVFSCSVMHEALHNHYTQKSLSLSLG

SEQ ID NO: 6 - protein, 218 aa, synthetic construct
  REGION 1..218: note = LC of PD1-3
EIVLTQSPATLSLSPGERATMSCRASENIDVSGISFMNWYQQKPGQAPKLLIYVASNQGSGIPARFSGSGSGTDFTLTISRLEPEDFAVYYCQQSKEVPWTFGQGTKLEIKRTVAAPSVFIFPPSDEQLKSGTASVVCLLNNFYPREAKVQWKVDNALQSGNSQESVTEQDSKDSTYSLSSTLTLSKADYEKHKVYACEVTHQGLSSPVTKSFNRGEC

SEQ ID NO: 7 - protein, 446 aa, synthetic construct; identical to SEQ ID NO: 5
  REGION 1..446: note = HC of PD1-4

SEQ ID NO: 8 - protein, 218 aa, synthetic construct; identical to SEQ ID NO: 6
  REGION 1..218: note = LC of PD1-4

SEQ ID NO: 9 - protein, 446 aa, synthetic construct; identical to SEQ ID NO: 5
  REGION 1..446: note = HC of PD1-5

SEQ ID NO: 10 - protein, 218 aa, synthetic construct; identical to SEQ ID NO: 6
  REGION 1..218: note = LC of PD1-5

SEQ ID NO: 11 - protein, 448 aa, synthetic construct
  REGION 1..448: note = HC of LAG3-1
QVTLVESGGGVVQPGRSLRLSCAFSGFSLSTSDMGVGWIRQAPGKGLEWVAHIWWDDVKRYNPALKSRFTISRDNSKNTLYLQMNSLRAEDTAVYFCARIEDYGVSYYFDYWGQGTTVTVSSASTKGPSVFPLAPCSRSTSESTAALGCLVKDYFPEPVTVSWNSGALTSGVHTFPAVLQSSGLYSLSSVVTVPSSSLGTKTYTCNVDHKPSNTKVDKRVESKYGPPCPPCPAPEFLGGPSVFLFPPKPKDTLMISRTPEVTCVVVDVSQEDPEVQFNWYVDGVEVHNAKTKPREEQFNSTYRVVSVLTVLHQDWLNGKEYKCKVSNKGLPSSIEKTISKAKGQPREPQVYTLPPSQEEMTKNQVSLTCLVKGFYPSDIAVEWESNGQPENNYKTTPPVLDSDGSFFLYSRLTVDKSRWQEGNVFSCSVMHEALHNHYTQKSLSLSLG

SEQ ID NO: 12 - protein, 214 aa, synthetic construct
  REGION 1..214: note = LC of LAG3-1
DIQMTQSPSFLSASVGDRVSITCKASQDVSTAVAWYQQKPGKAPKLLIYSASYRYTGVPDRFSGSGSGTDFTLTISSLQPEDFATYYCQQHYSIPLTFGQGTKLEIKRTVAAPSVFIFPPSDEQLKSGTASVVCLLNNFYPREAKVQWKVDNALQSGNSQESVTEQDSKDSTYSLSSTLTLSKADYEKHKVYACEVTHQGLSSPVTKSFNRGEC

SEQ ID NO: 13 - protein, 448 aa, synthetic construct
  REGION 1..448: note = HC of LAG3-2
QVTLKESGPTLVKPTQTLTLTCSFSGFSLSTSDMGVGWIRQPPGKALEWLAHIWWDDVKRYNPALKSRLTITKDTSKNQVVLTMTNMDPVDTATYFCARIEDYGVSYYFDYWGQGTTVTVSSASTKGPSVFPLAPCSRSTSESTAALGCLVKDYFPEPVTVSWNSGALTSGVHTFPAVLQSSGLYSLSSVVTVPSSSLGTKTYTCNVDHKPSNTKVDKRVESKYGPPCPPCPAPEFLGGPSVFLFPPKPKDTLMISRTPEVTCVVVDVSQEDPEVQFNWYVDGVEVHNAKTKPREEQFNSTYRVVSVLTVLHQDWLNGKEYKCKVSNKGLPSSIEKTISKAKGQPREPQVYTLPPSQEEMTKNQVSLTCLVKGFYPSDIAVEWESNGQPENNYKTTPPVLDSDGSFFLYSRLTVDKSRWQEGNVFSCSVMHEALHNHYTQKSLSLSLG

SEQ ID NO: 14 - protein, 214 aa, synthetic construct
  REGION 1..214: note = LC of LAG3-2
DIQMTQSPSFLSASVGDRVTFTCKASQDVSTAVAWYQQKPGKAPKLLIYSASYRYTGVPDRFSGSGSGTDFTLTISSLQPEDFATYYCQQHYSIPLTFGQGTKLEIKRTVAAPSVFIFPPSDEQLKSGTASVVCLLNNFYPREAKVQWKVDNALQSGNSQESVTEQDSKDSTYSLSSTLTLSKADYEKHKVYACEVTHQGLSSPVTKSFNRGEC

SEQ ID NO: 15 - protein, 448 aa, synthetic construct
  REGION 1..448: note = HC of LAG3-3
QVTLVESGGGVVQPGRSLSLSCAFSGFSLSTSDMGVGWVRQPPGKGLEWVAHIWWDDVKRYNPALKSRFTISRDNSKNTLYLQMNSLRAEDTATYYCARIEDYGVSYYFDYWGQGTTVTVSSASTKGPSVFPLAPCSRSTSESTAALGCLVKDYFPEPVTVSWNSGALTSGVHTFPAVLQSSGLYSLSSVVTVPSSSLGTKTYTCNVDHKPSNTKVDKRVESKYGPPCPPCPAPEFLGGPSVFLFPPKPKDTLMISRTPEVTCVVVDVSQEDPEVQFNWYVDGVEVHNAKTKPREEQFNSTYRVVSVLTVLHQDWLNGKEYKCKVSNKGLPSSIEKTISKAKGQPREPQVYTLPPSQEEMTKNQVSLTCLVKGFYPSDIAVEWESNGQPENNYKTTPPVLDSDGSFFLYSRLTVDKSRWQEGNVFSCSVMHEALHNHYTQKSLSLSLG

SEQ ID NO: 16 - protein, 214 aa, synthetic construct
  REGION 1..214: note = LC of LAG3-3
DIQMTQSPSFLSASVGDRVTITCKASQDVSTAVAWYQQKPGKAPKLLIYSASYRYTGVPDRFSGSGSGTDFTLTISSLQPEDFATYYCQQHYSIPLTFGAGTKLEIKRTVAAPSVFIFPPSDEQLKSGTASVVCLLNNFYPREAKVQWKVDNALQSGNSQESVTEQDSKDSTYSLSSTLTLSKADYEKHKVYACEVTHQGLSSPVTKSFNRGEC

SEQ ID NO: 17 - protein, 448 aa, synthetic construct
  REGION 1..448: note = HC of LAG3-4
QVTLVESGGGVVQPGRSLRLSCAFSGFSLSTSDMGVGWIRQAPGKGLEWVAHIWWDDVKRYNPALKSRFTISRDNSKNTLYLQMNSLRAEDTATYFCARIEDYGVSYYFDYWGQGTTVTVSSASTKGPSVFPLAPCSRSTSESTAALGCLVKDYFPEPVTVSWNSGALTSGVHTFPAVLQSSGLYSLSSVVTVPSSSLGTKTYTCNVDHKPSNTKVDKRVESKYGPPCPPCPAPEFLGGPSVFLFPPKPKDTLMISRTPEVTCVVVDVSQEDPEVQFNWYVDGVEVHNAKTKPREEQFNSTYRVVSVLTVLHQDWLNGKEYKCKVSNKGLPSSIEKTISKAKGQPREPQVYTLPPSQEEMTKNQVSLTCLVKGFYPSDIAVEWESNGQPENNYKTTPPVLDSDGSFFLYSRLTVDKSRWQEGNVFSCSVMHEALHNHYTQKSLSLSLG

SEQ ID NO: 18 - protein, 214 aa, synthetic construct
  REGION 1..214: note = LC of LAG3-4
DIVMTQSPSFLSASVGDRVTITCKASQDVSTAVAWYQQKPGKAPKLLIYSASYRYTGVPDRFSGSGSGTDFTLTISSLQPEDFATYYCQQHYSIPLTFGQGTKLEIKRTVAAPSVFIFPPSDEQLKSGTASVVCLLNNFYPREAKVQWKVDNALQSGNSQESVTEQDSKDSTYSLSSTLTLSKADYEKHKVYACEVTHQGLSSPVTKSFNRGEC

SEQ ID NO: 19 - protein, 448 aa, synthetic construct
  REGION 1..448: note = HC of LAG3-5
QVTLKESGPTLVKPTQTLTLTCSFSGFSLSTSDMGVGWIRQPPGKALEWLAHIWWDDVKRYNPALKSRLTITKDTSKNQVVLTMTNMDPVDTATYFCARIVDYGVSYYFDYWGQGTTVTVSSASTKGPSVFPLAPCSRSTSESTAALGCLVKDYFPEPVTVSWNSGALTSGVHTFPAVLQSSGLYSLSSVVTVPSSSLGTKTYTCNVDHKPSNTKVDKRVESKYGPPCPPCPAPEFLGGPSVFLFPPKPKDTLMISRTPEVTCVVVDVSQEDPEVQFNWYVDGVEVHNAKTKPREEQFNSTYRVVSVLTVLHQDWLNGKEYKCKVSNKGLPSSIEKTISKAKGQPREPQVYTLPPSQEEMTKNQVSLTCLVKGFYPSDIAVEWESNGQPENNYKTTPPVLDSDGSFFLYSRLTVDKSRWQEGNVFSCSVMHEALHNHYTQKSLSLSLG

SEQ ID NO: 20 - protein, 214 aa, synthetic construct
  REGION 1..214: note = LC of LAG3-5
DIQMTQSPSFLSASVGDRVSITCKASQDVSTAVAWYQQKPGKAPKLLIYSASYRYTGVPDRFSGSGSGTDFTLTISSLQPEDFAVYYCQQHYSIPLTFGQGTKLEIKRTVAAPSVFIFPPSDEQLKSGTASVVCLLNNFYPREAKVQWKVDNALQSGNSQESVTEQDSKDSTYSLSSTLTLSKADYEKHKVYACEVTHQGLSSPVTKSFNRGEC